European Patent Specification EP 3 831 953 B1, published December 13, 2023. Title: Paper-based detecting kit for nucleic acid and detecting method thereof. Applicant: THE ASAN FOUNDATION University of Ulsan Foundation For Industry Cooperation. The sequence listing filed with the application follows.

SEQUENCE LISTING (4 sequences)

SEQ ID NO: 1 - DNA, 31 bp, Artificial Sequence
  HPV 16 DNA forward primer
ttgttggggtaaccaactatttgttactgtt

SEQ ID NO: 2 - DNA, 29 bp, Artificial Sequence
  HPV 16 DNA reverse primer
cctccccatgtctgaggtactccttaaag

SEQ ID NO: 3 - DNA, 25 bp, Artificial Sequence
  HPV forward primer
tgtcagaaccatatggcgacagctt

SEQ ID NO: 4 - DNA, 25 bp, Artificial Sequence
  HPV reverse primer
ttcaccaacagcaccagccctatta